European Patent Specification EP 3 575 389 B1, published April 9, 2025. Title: CONSUMER PRODUCTS. Applicant: The Procter & Gamble Company. The sequence listing filed with the application follows.

SEQUENCE LISTING (77 sequences)

SEQ ID NO: 1 - protein, 269 aa, Bacillus lentus
AQSVPWGISRVQAPAAHNRGLTGSGVKVAVLDTGISTHPDLNIRGGASFVPGEPSTQDGNGHGTHVAGTIAALNNSIGVLGVAPSAELYAVKVLGASGSGSVSSIAQGLEWAGNNGMHVANLSLGSPSPSATLEQAVNSATSRGVLVVAASGNSGAGSISYPARYANAMAVGATDQNNNRASFSQYGAGLDIVAPGVNVQSTYPGSTYASLNGTSMATPHVAGAAALVKQKNPSWSNVQIRNHLKNTATSLGSTNLYGSGLVNAEAATR

SEQ ID NO: 2 - protein, 275 aa, BAcillus Amyloliquefaciens [sequence omitted]

SEQ ID NO: 3 - protein, 380 aa, Bacillus lentus
VRSKKLWIVASTALLISVAFSSSIASAAEEAKEKYLIGFNEQEAVSEFVEQVEANDEVAILSEEEEVEIELLHEFETIPVLSVELSPEDVDALELDPAISYIEEDAEVTTMAQSVPWGISRVQAPAAHNRGLTGSGVKVAVLDTGISTHPDLNIRGGASFVPGEPSTQDGNGHGTHVAGTIAALNNSIGVLGVAPSAELYAVKVLGASGSGSVSSIAQGLEWAGNNGMHVANLSLGSPSPSATLEQAVNSATSRGVLVVAASGNSGAGSISYPARYANAMAVGATDQNNNRASFSQYGAGLDIVAPGVNVQSTYPGSTYASLNGTSMATPHVAGAAALVKQKNPSWSNVQIRNHLKNTATSLGSTNLYGSGLVNAEAATR

SEQ ID NO: 4 - DNA, 1143 bp, Bacillus lentus
gtgagaagcaaaaaattgtggatcgtcgcgtcgaccgcactactcatttctgttgctttcagttcatcgatcgcatcggctgctgaagaagcaaaagaaaaatatttaattggctttaatgagcaggaagctgtcagtgagtttgtagaacaagtagaggcaaatgacgaggtcgccattctctctgaggaagaggaagtcgaaattgaattgcttcatgaatttgaaacgattcctgttttatccgttgagttaagcccagaagatgtggacgcgcttgagctcgatccagcgatttcttatattgaagaggatgcagaagtaacgacaatggcgcaatcagtgccatggggaattagccgtgtgcaagccccagctgcccataaccgtggattgacaggttctggtgtaaaagttgctgtcctcgatacaggtatttccactcatccagacttaaatattcgtggtggcgctagctttgtaccaggggaaccatccactcaagatgggaatgggcatggcacgcatgtggccgggacgattgctgctttaaacaattcgattggcgttcttggcgtagcgccgagcgcggaactatacgctgttaaagtattaggggcgagcggttcaggttcggtcagctcgattgcccaaggattggaatgggcagggaacaatggcatgcacgttgctaatttgagtttaggaagcccttcgccaagtgccacacttgagcaagctgttaatagcgcgacttctagaggcgttcttgttgtagcggcatctggaaattcaggtgcaggctcaatcagctatccggcccgttatgcgaacgcaatggcagtcggagctactgaccaaaacaacaaccgcgccagcttttcacagtatggcgcagggcttgacattgtcgcaccaggtgtaaacgtgcagagcacatacccaggttcaacgtatgccagcttaaacggtacatcgatggctactcctcatgttgcaggtgcagcagcccttgttaaacaaaagaacccatcttggtccaatgtacaaatccgcaatcatctaaagaatacggcaacgagcttaggaagcacgaacttgtatggaagcggacttgtcaatgcagaagctgcaactcgttaa

SEQ ID NO: 5 - DNA, 54 bp, Artificial Sequence
  Primer
aaagtattaggggcgagcggtgcaggtggacttagctcgattgcccaaggattg

SEQ ID NO: 6 - DNA, 46 bp, Artificial Sequence
  Primer
catctggaaattcaggtgcagaatcaatcagctatccggcccgtta

SEQ ID NO: 7 - DNA, 45 bp, Artificial Sequence
  Primer
ctgcccataaccgtggattggcaggttctggtgtaaaagttgctg

SEQ ID NO: 8 - DNA, 45 bp, Artificial Sequence; identical to SEQ ID NO: 7
  Primer

SEQ ID NO: 9 - DNA, 44 bp, Artificial Sequence
  Primer
gaagcggacttgtcaatgcattcgctgcaactcgttaaagcttg

SEQ ID NO: 10 - DNA, 48 bp, Artificial Sequence
  Primer
aaagtattaggggcgagcggtgcaggttcggtcagctcgattgcccaa

SEQ ID NO: 11 - DNA, 47 bp, Artificial Sequence
  Primer
tattaggggcgagcggttcaggtggagtcagctcgattgcccaagga

SEQ ID NO: 12 - DNA, 46 bp, Artificial Sequence
  Primer
gtcagctcgattgcccaaggagtagaatgggcagggaacaatggca

SEQ ID NO: 13 - DNA, 48 bp, Artificial Sequence
  Primer
cgttgctaatttgagtttaggaaacccttcgccaagtgccacacttga

SEQ ID NO: 14 - DNA, 42 bp, Artificial Sequence
  Primer
gaaccatccactcaagatggggaagggcatggcacgcatgtg

SEQ ID NO: 15 - DNA, 47 bp, Artificial Sequence
  Primer
accaaaacaacaaccgcgccgacttttcacagtatggcgcagggctt

SEQ ID NO: 16 - DNA, 23 bp, Artificial Sequence
  Primer
catatgagttatgcagtttgtag

SEQ ID NO: 17 - DNA, 23 bp, Artificial Sequence
  Primer
tgtttttcttggaattgtgctgt

SEQ ID NO: 18 - DNA, 23 bp, Artificial Sequence
  Primer
cagtttgtagaatgcaaaaagtg

SEQ ID NO: 19 - DNA, 23 bp, Artificial Sequence
  Primer
gacaaggtaaaggataaaacagc

SEQ ID NO: 20 - DNA, 40 bp, Artificial Sequence
  Primer
cataaccgtggattggcaggttctggtgtaaaagttgctg

SEQ ID NO: 21 - DNA, 40 bp, Artificial Sequence
  Primer
acttttacaccagaacctgccaatccacggttatgggcag

SEQ ID NO: 22 - DNA, 35 bp, Artificial Sequence
  Primer
cactcaagatggggaagggcatggcacgcatgtgg

SEQ ID NO: 23 - DNA, 39 bp, Artificial Sequence
  Primer
atgcgtgccatgcccttccccatcttgagtggatggttc

SEQ ID NO: 24 - DNA, 39 bp, Artificial Sequence
  Primer
gcgagcggttcaggtggagtcagctcgattgcccaagga

SEQ ID NO: 25 - DNA, 40 bp, Artificial Sequence
  Primer
tgggcaatcgagctgactccacctgaaccgctcgccccta

SEQ ID NO: 26 - DNA, 52 bp, Artificial Sequence
  Primer
gtggagtcagctcgattgcccaaggagtagaatgggcagggaacaatggcat

SEQ ID NO: 27 - DNA, 52 bp, Artificial Sequence
  Primer
cattctactccttgggcaatcgagctgactccacctgaaccgctcgccccta

SEQ ID NO: 28 - DNA, 42 bp, Artificial Sequence
  Primer
gcgagcggtggaggtgcgatcagctcgattgcccaaggattg

SEQ ID NO: 29 - DNA, 50 bp, Artificial Sequence
  Primer
cttgggcaatcgagctgatcgcacctccaccgctcgcccctaatacttta

SEQ ID NO: 30 - DNA, 42 bp, Artificial Sequence
  Primer
gcgagcggtgcaggtggacttagctcgattgcccaaggattg

SEQ ID NO: 31 - DNA, 50 bp, Artificial Sequence
  Primer
cttgggcaatcgagctaagtccacctgcaccgctcgcccctaatacttta

SEQ ID NO: 32 - DNA, 40 bp, Artificial Sequence
  Primer
tattaggggcgagcggtgcaggttcggtcagctcgattgc

SEQ ID NO: 33 - DNA, 42 bp, Artificial Sequence
  Primer
atcgagctgaccgaacctgcaccgctcgcccctaatacttta

SEQ ID NO: 34 - DNA, 41 bp, Artificial Sequence
  Primer
ctaatttgagtttaggaaacccttcgccaagtgccacactt

SEQ ID NO: 35 - DNA, 41 bp, Artificial Sequence
  Primer
gcacttggcgaagggtttcctaaactcaaattagcaacgtg

SEQ ID NO: 36 - DNA, 39 bp, Artificial Sequence
  Primer
gaaattcaggtgcagactcaatcagctatccggcccgtt

SEQ ID NO: 37 - DNA, 38 bp, Artificial Sequence
  Primer
ggatagctgattgagtctgcacctgaatttccagatgc

SEQ ID NO: 38 - DNA, 39 bp, Artificial Sequence
  Primer
gaaattcaggtgcagaatcaatcagctatccggcccgtt

SEQ ID NO: 39 - DNA, 38 bp, Artificial Sequence
  Primer
ggatagctgattgattctgcacctgaatttccagatgc

SEQ ID NO: 40 - DNA, 41 bp, Artificial Sequence
  Primer
aacgtgcagagcacagaaccaggttcaacgtatgccagctt

SEQ ID NO: 41 - DNA, 40 bp, Artificial Sequence
  Primer
catacgttgaacctggttctgtgctctgcacgtttacacc

SEQ ID NO: 42 - DNA, 41 bp, Artificial Sequence
  Primer
tcgattgcccaaggagtagaatgggcagggaacaatggcat

SEQ ID NO: 43 - DNA, 43 bp, Artificial Sequence
  Primer
cattgttccctgcccattctactccttgggcaatcgagctgac

SEQ ID NO: 44 - DNA, 810 bp, Bacillus lentus
gcgcaatcagtgccatggggaattagccgtgtgcaagccccggctgcccataaccgtggattgacaggttctggtgtaaaagttgctgtcctcgatacaggtatttccactcatccagacttaaatattcgtggtggcgctagctttgtaccaggggaaccatccactcaagatgggaatgggcatggcacgcatgtggccgggacgattgctgctctaaacaattcgattggcgtacttggcgtagcgccgagcgcggaactatacgctgttaaagtattaggggcgagcggtgggggcgccatcagctcgattgcccaaggattggaatgggcagggaacaatggcatgcacgttgctaatttgagtttaggaagcccttcgccaagtgccacacttgagcaagctgttaatagcgcgacttctaggggcgttcttgttgtagcggcatctggaaattcgggtgcagactcaatcagctatccggcccgttatgcgaacgcaatggcagtcggagctactgaccaaaacaacaaccgcgccagcttttcacagtatggcgcagggcttgacatcgtcgcaccaggtgtaaacgtgcagagcacatacccaggttcaacgtatgccagcttaaacggtacatcgatggctactcctcatgttgcaggtgcagcagtccttgttaaacataagaacccatcttggtccaatgtacgaatccgcgatcatctaaagaaaacggcaacgagcttaggaagcacgaacttgtatggaagcggacttgtcaatgccgaagctgcaactcgttaa

SEQ ID NO: 45 - protein, 269 aa, Bacillus lentus
AQSVPWGISRVQAPAAHNRGLTGSGVKVAVLDTGISTHPDLNIRGGASFVPGEPSTQDGNGHGTHVAGTIAALNNSIGVLGVAPSAELYAVKVLGASGGGAISSIAQGLEWAGNNGMHVANLSLGSPSPSATLEQAVNSATSRGVLVVAASGNSGADSISYPARYANAMAVGATDQNNNRASFSQYGAGLDIVAPGVNVQSTYPGSTYASLNGTSMATPHVAGAAVLVKHKNPSWSNVRIRDHLKKTATSLGSTNLYGSGLVNAEAATR

SEQ ID NO: 46 - DNA, 41 bp, Artificial Sequence
  Primer
gtattaggggcgagcggtggcggcgccatcagctcgattgc

SEQ ID NO: 47 - DNA, 41 bp, Artificial Sequence
  Primer
gcaatcgagctgatggcgccgccaccgctcgcccctaatac

SEQ ID NO: 48 - DNA, 40 bp, Artificial Sequence
  Primer
ggggcgagcggtgggggcggcatcagctcgattgcccaag

SEQ ID NO: 49 - DNA, 40 bp, Artificial Sequence
  Primer
cttgggcaatcgagctgatgccgcccccaccgctcgcccc

SEQ ID NO: 50 - DNA, 44 bp, Artificial Sequence
  Primer
gggcgagcggtgggggcgccgttagctcgattgcccaaggattg

SEQ ID NO: 51 - DNA, 44 bp, Artificial Sequence
  Primer
caatccttgggcaatcgagctaacggcgcccccaccgctcgccc

SEQ ID NO: 52 - DNA, 45 bp, Artificial Sequence
  Primer
gcatctggaaattcgggtgcaggctcaatcagctatccggcccgt

SEQ ID NO: 53 - DNA, 45 bp, Artificial Sequence
  Primer
acgggccggatagctgattgagcctgcacccgaatttccagatgc

SEQ ID NO: 54 - DNA, 43 bp, Artificial Sequence
  Primer
ctcatgttgcaggtgcagcagcacttgttaaacataagaaccc

SEQ ID NO: 55 - DNA, 43 bp, Artificial Sequence
  Primer
gggttcttatgtttaacaagtgctgctgcacctgcaacatgag

SEQ ID NO: 56 - DNA, 44 bp, Artificial Sequence
  Primer
gtgcagcagtccttgttaaacaaaagaacccatcttggtccaat

SEQ ID NO: 57 - DNA, 44 bp, Artificial Sequence
  Primer
attggaccaagatgggttcttttgtttaacaaggactgctgcac

SEQ ID NO: 58 - DNA, 44 bp, Artificial Sequence
  Primer
ccatcttggtccaatgtacaaatccgcgatcatctaaagaaaac

SEQ ID NO: 59 - DNA, 44 bp, Artificial Sequence
  Primer
gttttctttagatgatcgcggatttgtacattggaccaagatgg

SEQ ID NO: 60 - DNA, 43 bp, Artificial Sequence
  Primer
ggtccaatgtacgaatccgcaatcatctaaagaaaacggcaac

SEQ ID NO: 61 - DNA, 43 bp, Artificial Sequence
  Primer
gttgccgttttctttagatgattgcggattcgtacattggacc

SEQ ID NO: 62 - DNA, 43 bp, Artificial Sequence
  Primer
gaatccgcgatcatctaaagaatacggcaacgagcttaggaag

SEQ ID NO: 63 - DNA, 43 bp, Artificial Sequence
  Primer
cttcctaagctcgttgccgtattctttagatgatcgcggattc

SEQ ID NO: 64 - DNA, 807 bp, Bacillus lentus
gcgcaatcagtgccatggggaattagccgtgtgcaagccccggctgcccataaccgtggattgacaggttctggtgtaaaagttgctgtcctcgatacaggtatttccactcatccagacttaaatattcgtggtggcgctagctttgtaccaggggaaccatccactcaagatgggaatgggcatggcacgcatgtggccgggacgattgctgctctaaacaattcgattggcgtacttggcgtagcgccgagcgcggaactatacgctgttaaagtattaggggcgagcggtgggggcgccatcagctcgattgcccaaggattggaatgggcagggaacaatggcatgcacgttgctaatttgagtttaggaagcccttcgccaagtgccacacttgagcaagctgttaatagcgcgacttctaggggcgttcttgttgtagcggcatctggaaattcgggtgcagactcaatcagctatccggcccgttatgcgaacgcaatggcagtcggagctactgaccaaaacaacaaccgcgccagcttttcacagtatggcgcagggcttgacatcgtcgcaccaggtgtaaacgtgcagagcacatacccaggttcaacgtatgccagcttaaacggtacatcgatggctactcctcatgttgcaggtgcagcagtccttgttaaacaaaagaacccatcttggtccaatgtacgaatccgcgatcatctaaagaatacggcaacgagcttaggaagcacgaacttgtatggaagcggacttgtcaatgccgaagctgcaactcgt

SEQ ID NO: 65 - protein, 269 aa, Bacillus lentus
AQSVPWGISRVQAPAAHNRGLTGSGVKVAVLDTGISTHPDLNIRGGASFVPGEPSTQDGNGHGTHVAGTIAALNNSIGVLGVAPSAELYAVKVLGASGGGAISSIAQGLEWAGNNGMHVANLSLGSPSPSATLEQAVNSATSRGVLVVAASGNSGADSISYPARYANAMAVGATDQNNNRASFSQYGAGLDIVAPGVNVQSTYPGSTYASLNGTSMATPHVAGAAVLVKQKNPSWSNVRIRDHLKNTATSLGSTNLYGSGLVNAEAATR

SEQ ID NO: 66 - DNA, 38 bp, Artificial Sequence
  Primer
gtacgaatccgcgatagactaaagaatacggcaacgag

SEQ ID NO: 67 - DNA, 44 bp, Artificial Sequence
  Primer
gcggacttgtcaatgcctttgctgcaactcgttaaagcttacat

SEQ ID NO: 68 - DNA, 41 bp, Artificial Sequence
  Prinmer
ggaaattcgggtgcagaatcaatcagctatccggcccgtta

SEQ ID NO: 69 - DNA, 38 bp, Artificial Sequence
  Primer
ctggaaattcgggtgaagactcaatcagctatccggcc

SEQ ID NO: 70 - DNA, 51 bp, Artificial Sequence
  Primer
cggcatctggaaattcgggtgaaggctcaatcagctatccggcccgttatg

SEQ ID NO: 71 - DNA, 42 bp, Artificial Sequence
  Primer
cataaccgtggattggcaggttctggtgtaaaagttgctgtc

SEQ ID NO: 72 - DNA, 38 bp, Artificial Sequence
  Primer
tccactcaagatggggaagggcatggcacgcatgtggc

SEQ ID NO: 73 - DNA, 42 bp, Artificial Sequence
  Primer
cttgttaaacaaaagagaccatcttggtccaatgtacgaatc

SEQ ID NO: 74 - DNA, 42 bp, Artificial Sequence
  Primer
aatgtacgaatccgcagacatctaaagaatacggcaacgagc

SEQ ID NO: 75 - DNA, 43 bp, Artificial Sequence
  Primer
cgatcatctaaagaatagagcaacgagcttaggaagcacgaac

SEQ ID NO: 76 - DNA, 42 bp, Artificial Sequence
  Primer
gtggattgacaggtagaggtgtaaaagttgctgtcctcgata

SEQ ID NO: 77 - DNA, 43 bp, Artificial Sequence
  Primer
acgattgctgctctagataattcgattggcgtacttggcgtag